European Patent Specification EP 3 630 816 B1, published March 20, 2024. Title: POLYPEPTIDES ANTAGONIZING WNT SIGNALING IN TUMOR CELLS. Applicant: Boehringer Ingelheim International GmbH. The sequence listing filed with the application follows.

SEQUENCE LISTING (38 sequences)

SEQ ID NO: 1 - protein, 5 aa, Artificial Sequence
  CDR1 of F0129097A08
TYVMG

SEQ ID NO: 2 - protein, 17 aa, Artificial Sequence
  CDR2 of F0129097A08
AISWSGGSTYYADSVKG

SEQ ID NO: 3 - protein, 18 aa, Artificial Sequence
  CDR3 of F0129097A08
SRGTSTPSRASGVSRYDY

SEQ ID NO: 4 - protein, 5 aa, Artificial Sequence
  CDR1 of F0129093A02
RYAVA

SEQ ID NO: 5 - protein, 17 aa, Artificial Sequence
  CDR2 of F0129093A02
AITWSSGRIDYADSVKG

SEQ ID NO: 6 - protein, 20 aa, Artificial Sequence
  CDR3 of F0129093A02
DRRPRSTGRSGTGSPSTYDY

SEQ ID NO: 7 - protein, 5 aa, Artificial Sequence
  CDR1 of F0129046C10(E1A,N32G)
IGAMG

SEQ ID NO: 8 - protein, 16 aa, Artificial Sequence
  CDR2 of F0129046C10(E1A,N32G)
AVSSGGSTYYVDSVKG

SEQ ID NO: 9 - protein, 12 aa, Artificial Sequence
  CDR3 of F0129046C10(E1A,N32G)
ETGPYGPPKRDY

SEQ ID NO: 10 - protein, 5 aa, Artificial Sequence
  CDR1 of F0129046C10
INAMG

SEQ ID NO: 11 - protein, 127 aa, Artificial Sequence
  F0129097A08 (E1A, V23A) ISVD full sequence
AVQLVESGGGLVQPGGSLRLSCAASGRTFSTYVMGWFRQAPGKEREFVAAISWSGGSTYYADSVKGRFTISRDNSKNTVYLQMNSLRPEDTAVYYCAASRGTSTPSRASGVSRYDYWGQGTLVTVSS

SEQ ID NO: 12 - protein, 130 aa, Artificial Sequence
  F0129093A02 ISVD full sequence
EVQLVESGGGLVQPGGSLRLSCAASGLTFSRYAVAWFRQAPGKEREFVAAITWSSGRIDYADSVKGRFTISRDNSKNTVYLQMNSLRPEDTAVYYCAADRRPRSTGRSGTGSPSTYDYWGQGTLVTVSSA

SEQ ID NO: 13 - protein, 120 aa, Artificial Sequence
  F0129046C10(E1A,N32G) ISVD full sequence
AVQLVESGGGLVQPGGSLRLSCAASGSIFRIGAMGWYRQAPGKQRELVAAVSSGGSTYYVDSVKGRFTISRDNSKNTVYLQMNSLRPEDTAVYYCNRETGPYGPPKRDYWGQGTLVTVSS

SEQ ID NO: 14 - protein, 120 aa, Artificial Sequence
  F0129046C10 ISVD full sequence
EVQLVESGGGLVQPGGSLRLSCAASGSIFRINAMGWYRQAPGKQRELVAAVSSGGSTYYVDSVKGRFTISRDNSKNTVYLQMNSLRPEDTAVYYCNRETGPYGPPKRDYWGQGTLVTVSS

SEQ ID NO: 15 - protein, 5 aa, Artificial Sequence
  ALB11 CDR1
SFGMS

SEQ ID NO: 16 - protein, 17 aa, Artificial Sequence
  ALB11 CDR2
SISGSGSDTLYADSVKG

SEQ ID NO: 17 - protein, 6 aa, Artificial Sequence
  ALB11 CDR3
GGSLSR

SEQ ID NO: 18 - protein, 432 aa, Artificial Sequence
  F012900082 full sequence
EVQLVESGGGLVQPGGSLRLSCVASGRTFSTYVMGWFRQAPGKEREFVAAISWSGGSTYYADSVKGRFTISRDNSKNTVYLQMNSLRPEDTAVYYCAASRGTSTPSRASGVSRYDYWGQGTLVTVSSGGGGSGGGGSGGGGSGGGGSGGGGSGGGGSGGGGSEVQLVESGGGLVQPGNSLRLSCAASGFTFSSFGMSWVRQAPGKGLEWVSSISGSGSDTLYADSVKGRFTISRDNAKTTLYLQMNSLRPEDTAVYYCTIGGSLSRSSQGTLVTVSSGGGGSGGGGSGGGGSGGGGSGGGGSGGGGSGGGGSEVQLVESGGGLVQPGGSLRLSCAASGSIFRINAMGWYRQAPGKQRELVAAVSSGGSTYYVDSVKGRFTISRDNSKNTVYLQMNSLRPEDTAVYYCNRETGPYGPPKRDYWGQGTLVTVSS

SEQ ID NO: 19 - protein, 435 aa, Artificial Sequence
  F012900135 full sequence
AVQLVESGGGLVQPGGSLRLSCAASGSIFRIGAMGWYRQAPGKQRELVAAVSSGGSTYYVDSVKGRFTISRDNSKNTVYLQMNSLRPEDTAVYYCNRETGPYGPPKRDYWGQGTLVTVSSGGGGSGGGGSGGGGSGGGGSGGGGSGGGGSGGGGSEVQLVESGGGLVQPGNSLRLSCAASGFTFSSFGMSWVRQAPGKGLEWVSSISGSGSDTLYADSVKGRFTISRDNAKTTLYLQMNSLRPEDTAVYYCTIGGSLSRSSQGTLVTVSSGGGGSGGGGSGGGGSGGGGSGGGGSGGGGSGGGGSEVQLVESGGGLVQPGGSLRLSCAASGLTFSRYAVAWFRQAPGKEREFVAAITWSSGRIDYADSVKGRFTISRDNSKNTVYLQMNSLRPEDTAVYYCAADRRPRSTGRSGTGSPSTYDYWGQGTLVTVSSA

SEQ ID NO: 20 - protein, 433 aa, Artificial Sequence
  F012900141 full sequence
AVQLVESGGGLVQPGGSLRLSCAASGRTFSTYVMGWFRQAPGKEREFVAAISWSGGSTYYADSVKGRFTISRDNSKNTVYLQMNSLRPEDTAVYYCAASRGTSTPSRASGVSRYDYWGQGTLVTVSSGGGGSGGGGSGGGGSGGGGSGGGGSGGGGSGGGGSEVQLVESGGGLVQPGNSLRLSCAASGFTFSSFGMSWVRQAPGKGLEWVSSISGSGSDTLYADSVKGRFTISRDNAKTTLYLQMNSLRPEDTAVYYCTIGGSLSRSSQGTLVTVSSGGGGSGGGGSGGGGSGGGGSGGGGSGGGGSGGGGSEVQLVESGGGLVQPGGSLRLSCAASGSIFRIGAMGWYRQAPGKQRELVAAVSSGGSTYYVDSVKGRFTISRDNSKNTVYLQMNSLRPEDTAVYYCNRETGPYGPPKRDYWGQGTLVTVSSA

SEQ ID NO: 21 - protein, 115 aa, Artificial Sequence [sequence omitted]

SEQ ID NO: 22 - protein, 121 aa, Artificial Sequence
  F0129046C10(N32G)
EVQLVESGGGLVQPGGSLRLSCAASGSIFRIGAMGWYRQAPGKQRELVAAVSSGGSTYYVDSVKGRFTISRDNSKNTVYLQMNSLRPEDTAVYYCNRETGPYGPPKRDYWGQGTLVTVSSA

SEQ ID NO: 23 - protein, 127 aa, Artificial Sequence
  F0129097A08
EVQLVESGGGLVQPGGSLRLSCVASGRTFSTYVMGWFRQAPGKEREFVAAISWSGGSTYYADSVKGRFTISRDNSKNTVYLQMNSLRPEDTAVYYCAASRGTSTPSRASGVSRYDYWGQGTLVTVSS

SEQ ID NO: 24 - protein, 30 aa, Artificial Sequence
  FR1 of F0129097A08 (E1A, V23A)
AVQLVESGGGLVQPGGSLRLSCAASGRTFS

SEQ ID NO: 25 - protein, 14 aa, Artificial Sequence
  FR2 of F0129097A08
WFRQAPGKEREFVA

SEQ ID NO: 26 - protein, 32 aa, Artificial Sequence
  FR3 of F0129097A08
RFTISRDNSKNTVYLQMNSLRPEDTAVYYCAA

SEQ ID NO: 27 - protein, 11 aa, Artificial Sequence
  FR4 of F0129097A08
WGQGTLVTVSS

SEQ ID NO: 28 - protein, 30 aa, Artificial Sequence
  FR1 of F0129093A02
EVQLVESGGGLVQPGGSLRLSCAASGLTFS

SEQ ID NO: 29 - protein, 12 aa, Artificial Sequence
  FR4 of F0129093A02
WGQGTLVTVSSA

SEQ ID NO: 30 - protein, 30 aa, Artificial Sequence
  FR1 of F0129097A08
EVQLVESGGGLVQPGGSLRLSCVASGRTFS

SEQ ID NO: 31 - protein, 30 aa, Artificial Sequence
  FR1 of F0129046C10 (E1A, N32G)
AVQLVESGGGLVQPGGSLRLSCAASGSIFR

SEQ ID NO: 32 - protein, 14 aa, Artificial Sequence
  FR2 of F0129046C10
WYRQAPGKQRELVA

SEQ ID NO: 33 - protein, 32 aa, Artificial Sequence
  FR3 of F0129046C10
RFTISRDNSKNTVYLQMNSLRPEDTAVYYCNR

SEQ ID NO: 34 - protein, 30 aa, Artificial Sequence
  FR1 of F0129046C10
EVQLVESGGGLVQPGGSLRLSCAASGSIFR

SEQ ID NO: 35 - protein, 30 aa, Artificial Sequence
  FR1 of ALB11
EVQLVESGGGLVQPGNSLRLSCAASGFTFS

SEQ ID NO: 36 - protein, 14 aa, Artificial Sequence
  FR2 of ALB11
WVRQAPGKGLEWVS

SEQ ID NO: 37 - protein, 32 aa, Artificial Sequence
  FR3 of ALB11
RFTISRDNAKTTLYLQMNSLRPEDTAVYYCTI

SEQ ID NO: 38 - protein, 11 aa, Artificial Sequence
  FR4 of ALB11
SSQGTLVTVSS